European Patent Application EP 4 223 306 A2, published August 9, 2023. Title: Treatment of ciliopaties. Applicant: Ethris GmbH. Application EP. The sequence listing filed with the application follows.

SEQUENCE LISTING (14 sequences)

SEQ ID NO: 1 - RNA, 3546 nt, synthetic construct
  misc_feature 1..3546: note = CCDC40 sequence with CYBA 5 and 3 UTR (ETH031T09) - codon optimized sequence encoding a functional version of a human CCDC40 protein
  source 1..3546: mol_type = other RNA
gggagaccgcgcctagcagtgtcccagccgggttcgtgtcgccgccaccatggctgaacctggcggagccgccggaagatcccaccctgaagatggctctgccagcgagggcgagaaagagggcaacaacgagagccacatggtgtcccccccagagaaggacgacggccagaaaggcgaagaggccgtgggctctaccgagcaccctgaggaagtgaccacacaggccgaggccgccattgaagagggcgaggtggaaacagagggcgaagccgctgtggaaggcgaagaggaagccgtgtcttacggcgacgccgagagcgaggaagagtactactacaccgagacaagcagccccgagggccagatctctgccgccgataccacctacccctacttcagcccccctcaggaactgcctggggaagaggcctacgatagcgtgtccggcgaagctggcctgcagggctttcagcaggaagccacaggccctcccgagagccgggaaagaagagtgacaagccccgagcctagccacggcgtgctgggaccatctgagcagatgggccaagtgacctctggccctgctgtgggcagactgacaggcagcacagaggaacctcagggccaggtgctgcctatgggagtgcagcaccggttcagactgagccacggcagcgacatcgagagcagcgacctggaagagttcgtcagccaggaacccgtgatccctcctggcgtgccagatgcccatcccagggaaggcgatctgcccgtgttccaggaccagatccagcagccctctaccgaagagggggctatggccgagagagtggaaagcgagggctccgacgaagaagccgaggacgagggatctcagctggtggtgctggaccccgaccaccctctgatggtgcggtttcaggccgccctgaagaactacctgaaccggcagatcgagaagctgaaactggacctgcaggaactggtggtggccacaaagcagagcagagcccagagacaggaactgggcgtgaacctgtacgaggtgcagcagcatctggtgcatctgcagaagctgctggaaaagagccacgaccggcacgccatggccagctctgagcgcagacagaaagaggaagaactgcaggccgccagagccctgtacaccaagacatgcgccgctgccaacgaggaacggaagaagctggctgccctgcagaccgagatggaaaacctggctctgcacctgttctacatgcagaatatcgaccaggacatgcgggacgacatcagagtgatgacccaggtcgtgaagaaggccgagacagagagaatccgggccgagattgagaagaaaaagcaggacctgtacgtggaccagctgaccaccagggcccagcagctggaagaggatatcgccctgttcgaggcccagtacctggcccaggccgaagatacccggatcctgagaaaggccgtgtccgaggcctgcaccgagatcgatgccatcagcgtggaaaagcggcggatcatgcagcagtgggccagcagcctcgtgggcatgaagcacagagatgaggcccaccgggccgtgctggaagctctgagaggctgtcagcaccaggccaagagcaccgacggcgagatcgaggcctacaagaaatccatcatgaaggaagaggaaaagaacgagaaactggccagcatcctgaacagaaccgaaaccgaggccaccctgctgcagaaactgaccacccagtgcctgaccaaacaggtggccctgcagtcccagttcaacacctacagactgaccctgcaggacaccgaggacgccctgagtcaggatcagctggaacagatgattctgaccgaggaactgcaggctatccggcaggccattcagggggagctggaactgcggagaaagaccgacgccgccatcagagagaagctgcaggaacacatgaccagcaacaagaccaccaagtacttcaaccagctgattctgcgcctgcagaaagaaaagaccaacatgatgacacacctgagcaagatcaacggcgacattgcccagaccaccctggacatcacccacaccagcagcagactggacgcccaccagaaaaccctggtggaactggaccaggatgtgaagaaagtgaacgagctgatcaccaacagccagagcgagatcagccggcggaccatcctgatcgagagaaagcagggcctgatcaacttcctgaacaaacagctggaaagaatggtgtccgagctgggcggcgaggaagtgggacctctggaactggaaatcaagcggctgagcaagctgatcgacgagcacgacggcaaggccgtgcaggctcaagtgacatggctgcggctgcagcaggaaatggtcaaagtgacccaggaacaggaagaacagctggcctccctggacgccagcaagaaagaactgcacatcatggaacagaaaaagctgcgggtggaaagcaagatcgagcaggaaaaaaaagaacagaaagaaatcgagcaccacatgaaggacctggacaacgacctgaagaaactgaatatgctgatgaacaagaaccgctgctccagcgaagaactggaacagaacaacagagtgaccgagaacgagttcgtgcggagcctgaaggccagcgagcgggaaaccatcaagatgcaggacaagctgaaccagctgtccgaggaaaaagccacactgctgaaccagctggtggaagccgagcaccagatcatgctgtgggagaagaagatccagctggccaaagaaatgcggagcagcgtggacagcgagatcggccagaccgaaatcagagccatgaagggcgagatccaccggatgaaagtgcggctgggacagctgctgaaacagcaggaaaagatgatccgggccatggaactggccgtggccagacgggaaaccgtgacaacccaggctgagggccagcggaagatggacagaaaggccctgacccggaccgacttccaccacaagcagctggaactgaggcggaagatccgggacgtgcggaaggccaccgatgagtgcacaaagacagtgctggaactggaagagacacagcggaacgtgtcctccagcctgctggaaaaacaggaaaagctgagcgtgatccaggccgacttcgacaccctggaagctgacctgacaagactgggagccctgaaaagacagaacctgtccgagatcgtggcactgcagacccggctgaaacatctgcaggctgtgaaagagggacgctacgtgttcctgttcagatccaagcagtctctggtgctggaaagacagcggctggacaagcggctggcactgattgccaccatcctggatagagtgcgcgacgagtacccacagttccaggaagcactgcacaaggtgtcccagatgatcgccaacaagctggaatcccctggccccagctgacctcgccccggacctgccctcccgccaggtgcacccacctgcaataaatgcagcgaagccgggattcg

SEQ ID NO: 2 - RNA, 3063 nt, synthetic construct
  misc_feature 1..3063: note = CCDC39 sequence with CYBA UTRs (ETH047T04) - codon optimized sequence encoding a functional version of a human CCDC39 protein
  source 1..3063: mol_type = other RNA
gggagaccgcgcctagcagtgtcccagccgggttcgtgtcgccgccaccatgagcagcgagtttctggccgaactgcactgggaggacggcttcgctattcccgtggccaacgaggaaaacaagctgctggaagatcagctgagcaagctgaaggacgagagagcctctctgcaggacgagctgagagagtacgaggaacggatcaacagcatgaccagccacttcaagaacgtgaagcaagagctgagcatcacccagagcctgtgcaaggccagagagagagaaaccgagagcgaggaacacttcaaggctatcgcccagcgcgagctgggaagagtgaaggatgagatccagcggctggaaaacgagatggccagcatcctggaaaagaagtccgacaaagagaacggcatcttcaaggccacacagaagctggacggcctgaagtgccagatgaactgggatcagcaggccctggaagcctggctggaagagtctgcccacaaggattctgacgccctgacactgcagaagtacgcccagcaggacgacaacaagatccgggctctgaccctgcagctggaaagactgaccctggaatgcaaccagaagcggaagatcctggacaacgagctgaccgagacaatcagcgcccagctggaactggataaggccgctcaggacttcagaaagatccacaacgagcggcaagaactgatcaagcagtgggagaacaccatcgagcagatgcagaaacgcgacggcgacatcgacaactgcgccctggaactcgcccggatcaagcaagagacacgcgagaaagagaacctggtcaaagagaagatcaagttcctcgagtccgagatcggcaacaacaccgagttcgagaagcggatcagcgtggccgacagaaagctgctgaagtgcagaaccgcctaccaggaccacgagacaagccggattcagctcaagggcgagctggattctctgaaggccaccgtgaacagaaccagcagcgatctggaagccctgcggaagaacatcagcaagatcaagaaggacatccacgaggaaaccgccaggctgcagaaaacaaagaaccacaatgagatcatccagaccaagctgaaagagatcaccgaaaagaccatgagcgtggaagagaaggccacaaacctggaagatatgctcaaagaggaagagaaagacgtcaaagaggtggacgttcaactgaacctgattaagggcgtgctgttcaagaaggcccaagagctgcagaccgaaaccatgaaggaaaaggccgtcctgtctgagatcgagggcaccagatctagcctgaagcacctgaaccatcagctgcagaagctcgacttcgagacactgaagcagcaagagatcatgtacagccaggatttccacatccagcaggtcgagcggcggatgtctagactgaagggcgagatcaactccgaggaaaaacaggccctcgaggccaagatcgtggaactgagaaagagcctcgaagagaagaagtctacctgcggcctgctggaaacccagattaagaagctgcacaacgacctgtacttcatcaagaaagcccacagcaagaacagcgacgagaagcagagcctgatgaccaagatcaatgagctgaacctgttcatcgatcggagcgaaaaagagctggacaaggccaagggcttcaagcaggacctgatgatcgaggacaacctgctgaagctggaagtgaagcggaccagagagatgctgcacagcaaggccgaggaagtgctgtctctggaaaagcggaagcagcagctgtacaccgccatggaagagagaaccgaagagatcaaggtgcacaagaccatgctggcttcccagatcagatacgtggaccaagagcgcgagaacatctccaccgagtttagagagagactgtccaagatcgagaagctgaagaaccgctacgagatcctgaccgtcgtgatgctgcctcctgagggcgaagaggaaaagacccaggcctactacgtgatcaaggcagcccaagaaaaagaggaactccagagagaaggcgactgcctggacgccaagattaacaaggccgaaaaagaaatctacgccctcgagaacaccctgcaggtcctgaacagctgcaacaacaactacaagcagagcttcaagaaagtcacccctagctccgacgagtacgagctgaagattcagctggaagaacagaaaagagccgtggacgagaagtacagatacaagcagcggcagatcagagagctgcaagaggatatccagagcatggaaaacaccctggacgtgatcgagcacctggccaacaacgtgaaagagaagctgtccgagaaacaggcctacagctttcagctgtccaaagagacagaggaacagaagcccaaactggaacgcgtgaccaagcagtgcgccaagctgacaaaagagatccggctgctgaaagacaccaaggacgaaaccatggaagaacaagacatcaagctgcgcgagatgaagcagttccacaaagtgatcgacgagatgctggtggacatcattgaagagaacacagagatccgcatcatcctgcagacctattttcagcagagcggcctggaactgcctaccgcctctacaaagggcagcagacagagcagcagatcccctagccacacaagcctgagcgccagaagctctagaagcaccagcacctctaccagccagtccagcattaaggtgctggaactcaagttccccgccagctctagcctcgtgggaagcccttctagacctagcagcgcctctagcagctccagcaacgtgaagtccaagaaaagctccaagtgacctcgccccggacctgccctcccgccaggtgcacccacctgcaataaatgcagcgaagccgggattcgaaaaaaaaaaaaaaaaaaaaaaaaaaaaaaaaaaaaaaaaaaaaaaaaaaaaaaaaaaaaaaaaaaaaaaaaaaaaaaaaaaaaaaaaaaaaaaaaaaaaaaaaaaaaaaaaaaaaaaaa

SEQ ID NO: 3 - RNA, 1644 nt, synthetic construct
  misc_feature 1..1644: note = Codon optimized sequence encoding a functional version of a tdTomato protein
  source 1..1644: mol_type = other RNA
gggagacccaagctggctagcgtttaaacttaagcttggtaccgcgggcccgggatccaccggtcgccaccatggtgagcaagggcgaggaggtcatcaaagagttcatgcgcttcaaggtgcgcatggagggctccatgaacggccacgagttcgagatcgagggcgagggcgagggccgcccctacgagggcacccagaccgccaagctgaaggtgaccaagggcggccccctgcccttcgcctgggacatcctgtccccccagttcatgtacggctccaaggcgtacgtgaagcaccccgccgacatccccgattacaagaagctgtccttccccgagggcttcaagtgggagcgcgtgatgaacttcgaggacggcggtctggtgaccgtgacccaggactcctccctgcaggacggcacgctgatctacaaggtgaagatgcgcggcaccaacttcccccccgacggccccgtaatgcagaagaagaccatgggctgggaggcctccaccgagcgcctgtacccccgcgacggcgtgctgaagggcgagatccaccaggccctgaagctgaaggacggcggccactacctggtggagttcaagaccatctacatggccaagaagcccgtgcaactgcccggctactactacgtggacaccaagctggacatcacctcccacaacgaggactacaccatcgtggaacagtacgagcgctccgagggccgccaccacctgttcctggggcatggcaccggcagcaccggcagcggcagctccggcaccgcctcctccgaggacaacaacatggccgtcatcaaagagttcatgcgcttcaaggtgcgcatggagggctccatgaacggccacgagttcgagatcgagggcgagggcgagggccgcccctacgagggcacccagaccgccaagctgaaggtgaccaagggcggccccctgcccttcgcctgggacatcctgtccccccagttcatgtacggctccaaggcgtacgtgaagcaccccgccgacatccccgattacaagaagctgtccttccccgagggcttcaagtgggagcgcgtgatgaacttcgaggacggcggtctggtgaccgtgacccaggactcctccctgcaggacggcacgctgatctacaaggtgaagatgcgcggcaccaacttcccccccgacggccccgtaatgcagaagaagaccatgggctgggaggcctccaccgagcgcctgtacccccgcgacggcgtgctgaagggcgagatccaccaggccctgaagctgaaggacggcggccactacctggtggagttcaagaccatctacatggccaagaagcccgtgcaactgcccggctactactacgtggacaccaagctggacatcacctcccacaacgaggactacaccatcgtggaacagtacgagcgctccgagggccgccaccacctgttcctgtacggcatggacgagctgtacaagtaggcggccaattctgcagaaaaaaaaaaaaaaaaaaaaaaaaaaaaaaaaaaaaaaaaaaaaaaaaaaaaaaaaaaaaaaaaaaaaaaaaaaaaaaaaaaaaaaaaaaaaaaaaaaaaaaaaaaaaaaaaaaaaaaaagcggcc

SEQ ID NO: 4 - RNA, 1327 nt, synthetic construct
  misc_feature 1..1327: note = MCIDAS sequence with Ethris minimal 5 UTR and optional 3 UTR - codon optimized sequence encoding a functional version of a human MCIDAS protein
  source 1..1327: mol_type = other RNA
gggagacgccaccatgcaagcttgtggcggcggagctgctggaagaagggccttcgatagcatctgccccaaccggatgcttgcccttcctggtagagccctgctgtgcaagcctggcaagcccgagagaaagttcgcccctccaagaaagttcttccccggctgtactggcggcagccctgtgtctgtgtatgaggaccctcctgatgccgagcctacagctctgcctgctctgaccacaatcgacctgcaggatctggccgattgcagctctctgctgggatctgatgctcctcctggcggagatctggctgcctctcagaatcacagccaccagacagaggccgacttcaacctgcaagacttccgggacaccgtggacgacctgatcagcgatagcagcagcatgatgagccccactctggccagcggcgatttcccattcagcccctgtgacatcagccctttcggcccttgtctgagccctccactggatcctagagcactgcagagcccacctctgaggcctccagatgttcctccacctgagcagtactggaaagaggtggccgaccagaaccagagagcactgggcgacgctctggtggaaaacaaccagctgcacgtgaccctgacacagaagcaagaagagatcgccagcctgaaagaacggaatgtgcagctgaaagagctggcctccaggacaagacacctggccagtgtgctggacaagctgatgatcacccagagcagagattgcggagccgccgctgaaccttttctgctgaaggccaaggccaagagaagcctggaagaactggtgtctgccgccggacaggattgcgctgaagtggatgccatcctgcgcgagatcagcgagagatgtgatgaggccctgcagagcagggaccccaaaagacctagactgctgcccgagcctgccaacaccgataccagacctggaaatctgcacggcgccttcagaggcctgagaaccgattgctctagaagcgccctgaacctgagccacagcgaactcgaagaaggcggcagcttcagcacccggatcagaagccacagcaccatcagaaccctggcctttccacagggcaacgccttcacaatcagaaccgccaacggcggctacaagttcagatgggtgccaagctgagctagccaccgggcaatacgagctcaagccagtctcaaaaaaaaaaaaaaaaaaaaaaaaaaaaaaaaaaaaaaaaaaaaaaaaaaaaaaaaaaaaaaaaaaaaaaaaaaaaaaaaaaaaaaaaaaaaaaaaaaaaaaaaaaaaaaaaaaaaaaaa

SEQ ID NO: 5 - RNA, 3446 nt, synthetic construct
  misc_feature 1..3446: note = Sequence with Ethris minimal 5 UTR (ETH031T06) - codon optimized sequence encoding a functional version of a human CCDC40 protein
  source 1..3446: mol_type = other RNA
gggagacgccaccatggctgaacctggcggagccgccggaagatcccaccctgaagatggctctgccagcgagggcgagaaagagggcaacaacgagagccacatggtgtcccccccagagaaggacgacggccagaaaggcgaagaggccgtgggctctaccgagcaccctgaggaagtgaccacacaggccgaggccgccattgaagagggcgaggtggaaacagagggcgaagccgctgtggaaggcgaagaggaagccgtgtcttacggcgacgccgagagcgaggaagagtactactacaccgagacaagcagccccgagggccagatctctgccgccgataccacctacccctacttcagcccccctcaggaactgcctggggaagaggcctacgatagcgtgtccggcgaagctggcctgcagggctttcagcaggaagccacaggccctcccgagagccgggaaagaagagtgacaagccccgagcctagccacggcgtgctgggaccatctgagcagatgggccaagtgacctctggccctgctgtgggcagactgacaggcagcacagaggaacctcagggccaggtgctgcctatgggagtgcagcaccggttcagactgagccacggcagcgacatcgagagcagcgacctggaagagttcgtcagccaggaacccgtgatccctcctggcgtgccagatgcccatcccagggaaggcgatctgcccgtgttccaggaccagatccagcagccctctaccgaagagggggctatggccgagagagtggaaagcgagggctccgacgaagaagccgaggacgagggatctcagctggtggtgctggaccccgaccaccctctgatggtgcggtttcaggccgccctgaagaactacctgaaccggcagatcgagaagctgaaactggacctgcaggaactggtggtggccacaaagcagagcagagcccagagacaggaactgggcgtgaacctgtacgaggtgcagcagcatctggtgcatctgcagaagctgctggaaaagagccacgaccggcacgccatggccagctctgagcgcagacagaaagaggaagaactgcaggccgccagagccctgtacaccaagacatgcgccgctgccaacgaggaacggaagaagctggctgccctgcagaccgagatggaaaacctggctctgcacctgttctacatgcagaatatcgaccaggacatgcgggacgacatcagagtgatgacccaggtcgtgaagaaggccgagacagagagaatccgggccgagattgagaagaaaaagcaggacctgtacgtggaccagctgaccaccagggcccagcagctggaagaggatatcgccctgttcgaggcccagtacctggcccaggccgaagatacccggatcctgagaaaggccgtgtccgaggcctgcaccgagatcgatgccatcagcgtggaaaagcggcggatcatgcagcagtgggccagcagcctcgtgggcatgaagcacagagatgaggcccaccgggccgtgctggaagctctgagaggctgtcagcaccaggccaagagcaccgacggcgagatcgaggcctacaagaaatccatcatgaaggaagaggaaaagaacgagaaactggccagcatcctgaacagaaccgaaaccgaggccaccctgctgcagaaactgaccacccagtgcctgaccaaacaggtggccctgcagtcccagttcaacacctacagactgaccctgcaggacaccgaggacgccctgagtcaggatcagctggaacagatgattctgaccgaggaactgcaggctatccggcaggccattcagggggagctggaactgcggagaaagaccgacgccgccatcagagagaagctgcaggaacacatgaccagcaacaagaccaccaagtacttcaaccagctgattctgcgcctgcagaaagaaaagaccaacatgatgacacacctgagcaagatcaacggcgacattgcccagaccaccctggacatcacccacaccagcagcagactggacgcccaccagaaaaccctggtggaactggaccaggatgtgaagaaagtgaacgagctgatcaccaacagccagagcgagatcagccggcggaccatcctgatcgagagaaagcagggcctgatcaacttcctgaacaaacagctggaaagaatggtgtccgagctgggcggcgaggaagtgggacctctggaactggaaatcaagcggctgagcaagctgatcgacgagcacgacggcaaggccgtgcaggctcaagtgacatggctgcggctgcagcaggaaatggtcaaagtgacccaggaacaggaagaacagctggcctccctggacgccagcaagaaagaactgcacatcatggaacagaaaaagctgcgggtggaaagcaagatcgagcaggaaaaaaaagaacagaaagaaatcgagcaccacatgaaggacctggacaacgacctgaagaaactgaatatgctgatgaacaagaaccgctgctccagcgaagaactggaacagaacaacagagtgaccgagaacgagttcgtgcggagcctgaaggccagcgagcgggaaaccatcaagatgcaggacaagctgaaccagctgtccgaggaaaaagccacactgctgaaccagctggtggaagccgagcaccagatcatgctgtgggagaagaagatccagctggccaaagaaatgcggagcagcgtggacagcgagatcggccagaccgaaatcagagccatgaagggcgagatccaccggatgaaagtgcggctgggacagctgctgaaacagcaggaaaagatgatccgggccatggaactggccgtggccagacgggaaaccgtgacaacccaggctgagggccagcggaagatggacagaaaggccctgacccggaccgacttccaccacaagcagctggaactgaggcggaagatccgggacgtgcggaaggccaccgatgagtgcacaaagacagtgctggaactggaagagacacagcggaacgtgtcctccagcctgctggaaaaacaggaaaagctgagcgtgatccaggccgacttcgacaccctggaagctgacctgacaagactgggagccctgaaaagacagaacctgtccgagatcgtggcactgcagacccggctgaaacatctgcaggctgtgaaagagggacgctacgtgttcctgttcagatccaagcagtctctggtgctggaaagacagcggctggacaagcggctggcactgattgccaccatcctggatagagtgcgcgacgagtacccacagttccaggaagcactgcacaaggtgtcccagatgatcgccaacaagctggaatcccctggccccagctgattcg

SEQ ID NO: 6 - RNA, 3447 nt, synthetic construct
  misc_feature 1..3447: note = Sequence with TISU 5 UTR (ETH031T07) - codon optimized sequence encoding a functional version of a human CCDC40 protein
  source 1..3447: mol_type = other RNA
gggagactgccaagatggctgaacctggcggagccgccggaagatcccaccctgaagatggctctgccagcgagggcgagaaagagggcaacaacgagagccacatggtgtcccccccagagaaggacgacggccagaaaggcgaagaggccgtgggctctaccgagcaccctgaggaagtgaccacacaggccgaggccgccattgaagagggcgaggtggaaacagagggcgaagccgctgtggaaggcgaagaggaagccgtgtcttacggcgacgccgagagcgaggaagagtactactacaccgagacaagcagccccgagggccagatctctgccgccgataccacctacccctacttcagcccccctcaggaactgcctggggaagaggcctacgatagcgtgtccggcgaagctggcctgcagggctttcagcaggaagccacaggccctcccgagagccgggaaagaagagtgacaagccccgagcctagccacggcgtgctgggaccatctgagcagatgggccaagtgacctctggccctgctgtgggcagactgacaggcagcacagaggaacctcagggccaggtgctgcctatgggagtgcagcaccggttcagactgagccacggcagcgacatcgagagcagcgacctggaagagttcgtcagccaggaacccgtgatccctcctggcgtgccagatgcccatcccagggaaggcgatctgcccgtgttccaggaccagatccagcagccctctaccgaagagggggctatggccgagagagtggaaagcgagggctccgacgaagaagccgaggacgagggatctcagctggtggtgctggaccccgaccaccctctgatggtgcggtttcaggccgccctgaagaactacctgaaccggcagatcgagaagctgaaactggacctgcaggaactggtggtggccacaaagcagagcagagcccagagacaggaactgggcgtgaacctgtacgaggtgcagcagcatctggtgcatctgcagaagctgctggaaaagagccacgaccggcacgccatggccagctctgagcgcagacagaaagaggaagaactgcaggccgccagagccctgtacaccaagacatgcgccgctgccaacgaggaacggaagaagctggctgccctgcagaccgagatggaaaacctggctctgcacctgttctacatgcagaatatcgaccaggacatgcgggacgacatcagagtgatgacccaggtcgtgaagaaggccgagacagagagaatccgggccgagattgagaagaaaaagcaggacctgtacgtggaccagctgaccaccagggcccagcagctggaagaggatatcgccctgttcgaggcccagtacctggcccaggccgaagatacccggatcctgagaaaggccgtgtccgaggcctgcaccgagatcgatgccatcagcgtggaaaagcggcggatcatgcagcagtgggccagcagcctcgtgggcatgaagcacagagatgaggcccaccgggccgtgctggaagctctgagaggctgtcagcaccaggccaagagcaccgacggcgagatcgaggcctacaagaaatccatcatgaaggaagaggaaaagaacgagaaactggccagcatcctgaacagaaccgaaaccgaggccaccctgctgcagaaactgaccacccagtgcctgaccaaacaggtggccctgcagtcccagttcaacacctacagactgaccctgcaggacaccgaggacgccctgagtcaggatcagctggaacagatgattctgaccgaggaactgcaggctatccggcaggccattcagggggagctggaactgcggagaaagaccgacgccgccatcagagagaagctgcaggaacacatgaccagcaacaagaccaccaagtacttcaaccagctgattctgcgcctgcagaaagaaaagaccaacatgatgacacacctgagcaagatcaacggcgacattgcccagaccaccctggacatcacccacaccagcagcagactggacgcccaccagaaaaccctggtggaactggaccaggatgtgaagaaagtgaacgagctgatcaccaacagccagagcgagatcagccggcggaccatcctgatcgagagaaagcagggcctgatcaacttcctgaacaaacagctggaaagaatggtgtccgagctgggcggcgaggaagtgggacctctggaactggaaatcaagcggctgagcaagctgatcgacgagcacgacggcaaggccgtgcaggctcaagtgacatggctgcggctgcagcaggaaatggtcaaagtgacccaggaacaggaagaacagctggcctccctggacgccagcaagaaagaactgcacatcatggaacagaaaaagctgcgggtggaaagcaagatcgagcaggaaaaaaaagaacagaaagaaatcgagcaccacatgaaggacctggacaacgacctgaagaaactgaatatgctgatgaacaagaaccgctgctccagcgaagaactggaacagaacaacagagtgaccgagaacgagttcgtgcggagcctgaaggccagcgagcgggaaaccatcaagatgcaggacaagctgaaccagctgtccgaggaaaaagccacactgctgaaccagctggtggaagccgagcaccagatcatgctgtgggagaagaagatccagctggccaaagaaatgcggagcagcgtggacagcgagatcggccagaccgaaatcagagccatgaagggcgagatccaccggatgaaagtgcggctgggacagctgctgaaacagcaggaaaagatgatccgggccatggaactggccgtggccagacgggaaaccgtgacaacccaggctgagggccagcggaagatggacagaaaggccctgacccggaccgacttccaccacaagcagctggaactgaggcggaagatccgggacgtgcggaaggccaccgatgagtgcacaaagacagtgctggaactggaagagacacagcggaacgtgtcctccagcctgctggaaaaacaggaaaagctgagcgtgatccaggccgacttcgacaccctggaagctgacctgacaagactgggagccctgaaaagacagaacctgtccgagatcgtggcactgcagacccggctgaaacatctgcaggctgtgaaagagggacgctacgtgttcctgttcagatccaagcagtctctggtgctggaaagacagcggctggacaagcggctggcactgattgccaccatcctggatagagtgcgcgacgagtacccacagttccaggaagcactgcacaaggtgtcccagatgatcgccaacaagctggaatcccctggccccagctgattcg

SEQ ID NO: 7 - RNA, 3476 nt, synthetic construct
  misc_feature 1..3476: note = Sequence with hAg 5 UTR but without 3 UTR (ETH031T08) - codon optimized sequence encoding a functional version of a human CCDC40 protein
  source 1..3476: mol_type = other RNA
gggagactcttctggtccccacagactcagagagaacgccaccatggctgaacctggcggagccgccggaagatcccaccctgaagatggctctgccagcgagggcgagaaagagggcaacaacgagagccacatggtgtcccccccagagaaggacgacggccagaaaggcgaagaggccgtgggctctaccgagcaccctgaggaagtgaccacacaggccgaggccgccattgaagagggcgaggtggaaacagagggcgaagccgctgtggaaggcgaagaggaagccgtgtcttacggcgacgccgagagcgaggaagagtactactacaccgagacaagcagccccgagggccagatctctgccgccgataccacctacccctacttcagcccccctcaggaactgcctggggaagaggcctacgatagcgtgtccggcgaagctggcctgcagggctttcagcaggaagccacaggccctcccgagagccgggaaagaagagtgacaagccccgagcctagccacggcgtgctgggaccatctgagcagatgggccaagtgacctctggccctgctgtgggcagactgacaggcagcacagaggaacctcagggccaggtgctgcctatgggagtgcagcaccggttcagactgagccacggcagcgacatcgagagcagcgacctggaagagttcgtcagccaggaacccgtgatccctcctggcgtgccagatgcccatcccagggaaggcgatctgcccgtgttccaggaccagatccagcagccctctaccgaagagggggctatggccgagagagtggaaagcgagggctccgacgaagaagccgaggacgagggatctcagctggtggtgctggaccccgaccaccctctgatggtgcggtttcaggccgccctgaagaactacctgaaccggcagatcgagaagctgaaactggacctgcaggaactggtggtggccacaaagcagagcagagcccagagacaggaactgggcgtgaacctgtacgaggtgcagcagcatctggtgcatctgcagaagctgctggaaaagagccacgaccggcacgccatggccagctctgagcgcagacagaaagaggaagaactgcaggccgccagagccctgtacaccaagacatgcgccgctgccaacgaggaacggaagaagctggctgccctgcagaccgagatggaaaacctggctctgcacctgttctacatgcagaatatcgaccaggacatgcgggacgacatcagagtgatgacccaggtcgtgaagaaggccgagacagagagaatccgggccgagattgagaagaaaaagcaggacctgtacgtggaccagctgaccaccagggcccagcagctggaagaggatatcgccctgttcgaggcccagtacctggcccaggccgaagatacccggatcctgagaaaggccgtgtccgaggcctgcaccgagatcgatgccatcagcgtggaaaagcggcggatcatgcagcagtgggccagcagcctcgtgggcatgaagcacagagatgaggcccaccgggccgtgctggaagctctgagaggctgtcagcaccaggccaagagcaccgacggcgagatcgaggcctacaagaaatccatcatgaaggaagaggaaaagaacgagaaactggccagcatcctgaacagaaccgaaaccgaggccaccctgctgcagaaactgaccacccagtgcctgaccaaacaggtggccctgcagtcccagttcaacacctacagactgaccctgcaggacaccgaggacgccctgagtcaggatcagctggaacagatgattctgaccgaggaactgcaggctatccggcaggccattcagggggagctggaactgcggagaaagaccgacgccgccatcagagagaagctgcaggaacacatgaccagcaacaagaccaccaagtacttcaaccagctgattctgcgcctgcagaaagaaaagaccaacatgatgacacacctgagcaagatcaacggcgacattgcccagaccaccctggacatcacccacaccagcagcagactggacgcccaccagaaaaccctggtggaactggaccaggatgtgaagaaagtgaacgagctgatcaccaacagccagagcgagatcagccggcggaccatcctgatcgagagaaagcagggcctgatcaacttcctgaacaaacagctggaaagaatggtgtccgagctgggcggcgaggaagtgggacctctggaactggaaatcaagcggctgagcaagctgatcgacgagcacgacggcaaggccgtgcaggctcaagtgacatggctgcggctgcagcaggaaatggtcaaagtgacccaggaacaggaagaacagctggcctccctggacgccagcaagaaagaactgcacatcatggaacagaaaaagctgcgggtggaaagcaagatcgagcaggaaaaaaaagaacagaaagaaatcgagcaccacatgaaggacctggacaacgacctgaagaaactgaatatgctgatgaacaagaaccgctgctccagcgaagaactggaacagaacaacagagtgaccgagaacgagttcgtgcggagcctgaaggccagcgagcgggaaaccatcaagatgcaggacaagctgaaccagctgtccgaggaaaaagccacactgctgaaccagctggtggaagccgagcaccagatcatgctgtgggagaagaagatccagctggccaaagaaatgcggagcagcgtggacagcgagatcggccagaccgaaatcagagccatgaagggcgagatccaccggatgaaagtgcggctgggacagctgctgaaacagcaggaaaagatgatccgggccatggaactggccgtggccagacgggaaaccgtgacaacccaggctgagggccagcggaagatggacagaaaggccctgacccggaccgacttccaccacaagcagctggaactgaggcggaagatccgggacgtgcggaaggccaccgatgagtgcacaaagacagtgctggaactggaagagacacagcggaacgtgtcctccagcctgctggaaaaacaggaaaagctgagcgtgatccaggccgacttcgacaccctggaagctgacctgacaagactgggagccctgaaaagacagaacctgtccgagatcgtggcactgcagacccggctgaaacatctgcaggctgtgaaagagggacgctacgtgttcctgttcagatccaagcagtctctggtgctggaaagacagcggctggacaagcggctggcactgattgccaccatcctggatagagtgcgcgacgagtacccacagttccaggaagcactgcacaaggtgtcccagatgatcgccaacaagctggaatcccctggccccagctgattcg

SEQ ID NO: 8 - RNA, 3683 nt, synthetic construct
  misc_feature 1..3683: note = Sequence with human CMV IE9 5 UTR and human Growth hormone 3 UTR (ETH031T10) - codon optimized sequence encoding a functional version of a human CCDC40 protein
  source 1..3683: mol_type = other RNA
gggagaccagatcgcctggagacgccatccacgctgttttgacctccatagaagacaccgggaccgatccagcctccgcggccgggaacggtgcattggaacgcggattccccgtgccaagagtgactcaccgtccttgacacggccaccatggctgaacctggcggagccgccggaagatcccaccctgaagatggctctgccagcgagggcgagaaagagggcaacaacgagagccacatggtgtcccccccagagaaggacgacggccagaaaggcgaagaggccgtgggctctaccgagcaccctgaggaagtgaccacacaggccgaggccgccattgaagagggcgaggtggaaacagagggcgaagccgctgtggaaggcgaagaggaagccgtgtcttacggcgacgccgagagcgaggaagagtactactacaccgagacaagcagccccgagggccagatctctgccgccgataccacctacccctacttcagcccccctcaggaactgcctggggaagaggcctacgatagcgtgtccggcgaagctggcctgcagggctttcagcaggaagccacaggccctcccgagagccgggaaagaagagtgacaagccccgagcctagccacggcgtgctgggaccatctgagcagatgggccaagtgacctctggccctgctgtgggcagactgacaggcagcacagaggaacctcagggccaggtgctgcctatgggagtgcagcaccggttcagactgagccacggcagcgacatcgagagcagcgacctggaagagttcgtcagccaggaacccgtgatccctcctggcgtgccagatgcccatcccagggaaggcgatctgcccgtgttccaggaccagatccagcagccctctaccgaagagggggctatggccgagagagtggaaagcgagggctccgacgaagaagccgaggacgagggatctcagctggtggtgctggaccccgaccaccctctgatggtgcggtttcaggccgccctgaagaactacctgaaccggcagatcgagaagctgaaactggacctgcaggaactggtggtggccacaaagcagagcagagcccagagacaggaactgggcgtgaacctgtacgaggtgcagcagcatctggtgcatctgcagaagctgctggaaaagagccacgaccggcacgccatggccagctctgagcgcagacagaaagaggaagaactgcaggccgccagagccctgtacaccaagacatgcgccgctgccaacgaggaacggaagaagctggctgccctgcagaccgagatggaaaacctggctctgcacctgttctacatgcagaatatcgaccaggacatgcgggacgacatcagagtgatgacccaggtcgtgaagaaggccgagacagagagaatccgggccgagattgagaagaaaaagcaggacctgtacgtggaccagctgaccaccagggcccagcagctggaagaggatatcgccctgttcgaggcccagtacctggcccaggccgaagatacccggatcctgagaaaggccgtgtccgaggcctgcaccgagatcgatgccatcagcgtggaaaagcggcggatcatgcagcagtgggccagcagcctcgtgggcatgaagcacagagatgaggcccaccgggccgtgctggaagctctgagaggctgtcagcaccaggccaagagcaccgacggcgagatcgaggcctacaagaaatccatcatgaaggaagaggaaaagaacgagaaactggccagcatcctgaacagaaccgaaaccgaggccaccctgctgcagaaactgaccacccagtgcctgaccaaacaggtggccctgcagtcccagttcaacacctacagactgaccctgcaggacaccgaggacgccctgagtcaggatcagctggaacagatgattctgaccgaggaactgcaggctatccggcaggccattcagggggagctggaactgcggagaaagaccgacgccgccatcagagagaagctgcaggaacacatgaccagcaacaagaccaccaagtacttcaaccagctgattctgcgcctgcagaaagaaaagaccaacatgatgacacacctgagcaagatcaacggcgacattgcccagaccaccctggacatcacccacaccagcagcagactggacgcccaccagaaaaccctggtggaactggaccaggatgtgaagaaagtgaacgagctgatcaccaacagccagagcgagatcagccggcggaccatcctgatcgagagaaagcagggcctgatcaacttcctgaacaaacagctggaaagaatggtgtccgagctgggcggcgaggaagtgggacctctggaactggaaatcaagcggctgagcaagctgatcgacgagcacgacggcaaggccgtgcaggctcaagtgacatggctgcggctgcagcaggaaatggtcaaagtgacccaggaacaggaagaacagctggcctccctggacgccagcaagaaagaactgcacatcatggaacagaaaaagctgcgggtggaaagcaagatcgagcaggaaaaaaaagaacagaaagaaatcgagcaccacatgaaggacctggacaacgacctgaagaaactgaatatgctgatgaacaagaaccgctgctccagcgaagaactggaacagaacaacagagtgaccgagaacgagttcgtgcggagcctgaaggccagcgagcgggaaaccatcaagatgcaggacaagctgaaccagctgtccgaggaaaaagccacactgctgaaccagctggtggaagccgagcaccagatcatgctgtgggagaagaagatccagctggccaaagaaatgcggagcagcgtggacagcgagatcggccagaccgaaatcagagccatgaagggcgagatccaccggatgaaagtgcggctgggacagctgctgaaacagcaggaaaagatgatccgggccatggaactggccgtggccagacgggaaaccgtgacaacccaggctgagggccagcggaagatggacagaaaggccctgacccggaccgacttccaccacaagcagctggaactgaggcggaagatccgggacgtgcggaaggccaccgatgagtgcacaaagacagtgctggaactggaagagacacagcggaacgtgtcctccagcctgctggaaaaacaggaaaagctgagcgtgatccaggccgacttcgacaccctggaagctgacctgacaagactgggagccctgaaaagacagaacctgtccgagatcgtggcactgcagacccggctgaaacatctgcaggctgtgaaagagggacgctacgtgttcctgttcagatccaagcagtctctggtgctggaaagacagcggctggacaagcggctggcactgattgccaccatcctggatagagtgcgcgacgagtacccacagttccaggaagcactgcacaaggtgtcccagatgatcgccaacaagctggaatcccctggccccagctgacgggtggcatccctgtgacccctccccagtgcctctcctggccctggaagttgccactccagtgcccaccagccttgtcctaataaaattaagttgcatcttcg

SEQ ID NO: 9 - RNA, 4295 nt, synthetic construct
  misc_feature 1..4295: note = ETH031T28: N terminal EGFP tag-CCDC40 - codon optimized sequence encoding a functional version of a human CCDC40 protein
  source 1..4295: mol_type = other RNA
gggagacgccaccatggtgagcaagggcgaggagctgttcaccggggtggtgcccatcctggtcgagctggacggcgacgtaaacggccacaagttcagcgtgtccggcgagggcgagggcgatgccacctacggcaagctgaccctgaagttcatctgcaccaccggcaagctgcccgtgccctggcccaccctcgtgaccaccctgacctacggcgtgcagtgcttcagccgctaccccgaccacatgaagcagcacgacttcttcaagtccgccatgcccgaaggctacgtccaggagcgcaccatcttcttcaaggacgacggcaactacaagacccgcgccgaggtgaagttcgagggcgacaccctggtgaaccgcatcgagctgaagggcatcgacttcaaggaggacggcaacatcctggggcacaagctggagtacaactacaacagccacaacgtctatatcatggccgacaagcagaagaacggcatcaaggtgaacttcaagatccgccacaacatcgaggacggcagcgtgcagctcgccgaccactaccagcagaacacccccatcggcgacggccccgtgctgctgcccgacaaccactacctgagcacccagtccgccctgagcaaagaccccaacgagaagcgcgatcacatggtcctgctggagttcgtgaccgccgccgggatcactctcggcatggacgagctgtacaagggcggagggggcagcgctgaacctggcggagccgccggaagatcccaccctgaagatggctctgccagcgagggcgagaaagagggcaacaacgagagccacatggtgtcccccccagagaaggacgacggccagaaaggcgaagaggccgtgggctctaccgagcaccctgaggaagtgaccacacaggccgaggccgccattgaagagggcgaggtggaaacagagggcgaagccgctgtggaaggcgaagaggaagccgtgtcttacggcgacgccgagagcgaggaagagtactactacaccgagacaagcagccccgagggccagatctctgccgccgataccacctacccctacttcagcccccctcaggaactgcctggggaagaggcctacgatagcgtgtccggcgaagctggcctgcagggctttcagcaggaagccacaggccctcccgagagccgggaaagaagagtgacaagccccgagcctagccacggcgtgctgggaccatctgagcagatgggccaagtgacctctggccctgctgtgggcagactgacaggcagcacagaggaacctcagggccaggtgctgcctatgggagtgcagcaccggttcagactgagccacggcagcgacatcgagagcagcgacctggaagagttcgtcagccaggaacccgtgatccctcctggcgtgccagatgcccatcccagggaaggcgatctgcccgtgttccaggaccagatccagcagccctctaccgaagagggggctatggccgagagagtggaaagcgagggctccgacgaagaagccgaggacgagggatctcagctggtggtgctggaccccgaccaccctctgatggtgcggtttcaggccgccctgaagaactacctgaaccggcagatcgagaagctgaaactggacctgcaggaactggtggtggccacaaagcagagcagagcccagagacaggaactgggcgtgaacctgtacgaggtgcagcagcatctggtgcatctgcagaagctgctggaaaagagccacgaccggcacgccatggccagctctgagcgcagacagaaagaggaagaactgcaggccgccagagccctgtacaccaagacatgcgccgctgccaacgaggaacggaagaagctggctgccctgcagaccgagatggaaaacctggctctgcacctgttctacatgcagaatatcgaccaggacatgcgggacgacatcagagtgatgacccaggtcgtgaagaaggccgagacagagagaatccgggccgagattgagaagaaaaagcaggacctgtacgtggaccagctgaccaccagggcccagcagctggaagaggatatcgccctgttcgaggcccagtacctggcccaggccgaagatacccggatcctgagaaaggccgtgtccgaggcctgcaccgagatcgatgccatcagcgtggaaaagcggcggatcatgcagcagtgggccagcagcctcgtgggcatgaagcacagagatgaggcccaccgggccgtgctggaagctctgagaggctgtcagcaccaggccaagagcaccgacggcgagatcgaggcctacaagaaatccatcatgaaggaagaggaaaagaacgagaaactggccagcatcctgaacagaaccgaaaccgaggccaccctgctgcagaaactgaccacccagtgcctgaccaaacaggtggccctgcagtcccagttcaacacctacagactgaccctgcaggacaccgaggacgccctgagtcaggatcagctggaacagatgattctgaccgaggaactgcaggctatccggcaggccattcagggggagctggaactgcggagaaagaccgacgccgccatcagagagaagctgcaggaacacatgaccagcaacaagaccaccaagtacttcaaccagctgattctgcgcctgcagaaagaaaagaccaacatgatgacacacctgagcaagatcaacggcgacattgcccagaccaccctggacatcacccacaccagcagcagactggacgcccaccagaaaaccctggtggaactggaccaggatgtgaagaaagtgaacgagctgatcaccaacagccagagcgagatcagccggcggaccatcctgatcgagagaaagcagggcctgatcaacttcctgaacaaacagctggaaagaatggtgtccgagctgggcggcgaggaagtgggacctctggaactggaaatcaagcggctgagcaagctgatcgacgagcacgacggcaaggccgtgcaggctcaagtgacatggctgcggctgcagcaggaaatggtcaaagtgacccaggaacaggaagaacagctggcctccctggacgccagcaagaaagaactgcacatcatggaacagaaaaagctgcgggtggaaagcaagatcgagcaggaaaaaaaagaacagaaagaaatcgagcaccacatgaaggacctggacaacgacctgaagaaactgaatatgctgatgaacaagaaccgctgctccagcgaagaactggaacagaacaacagagtgaccgagaacgagttcgtgcggagcctgaaggccagcgagcgggaaaccatcaagatgcaggacaagctgaaccagctgtccgaggaaaaagccacactgctgaaccagctggtggaagccgagcaccagatcatgctgtgggagaagaagatccagctggccaaagaaatgcggagcagcgtggacagcgagatcggccagaccgaaatcagagccatgaagggcgagatccaccggatgaaagtgcggctgggacagctgctgaaacagcaggaaaagatgatccgggccatggaactggccgtggccagacgggaaaccgtgacaacccaggctgagggccagcggaagatggacagaaaggccctgacccggaccgacttccaccacaagcagctggaactgaggcggaagatccgggacgtgcggaaggccaccgatgagtgcacaaagacagtgctggaactggaagagacacagcggaacgtgtcctccagcctgctggaaaaacaggaaaagctgagcgtgatccaggccgacttcgacaccctggaagctgacctgacaagactgggagccctgaaaagacagaacctgtccgagatcgtggcactgcagacccggctgaaacatctgcaggctgtgaaagagggacgctacgtgttcctgttcagatccaagcagtctctggtgctggaaagacagcggctggacaagcggctggcactgattgccaccatcctggatagagtgcgcgacgagtacccacagttccaggaagcactgcacaaggtgtcccagatgatcgccaacaagctggaatcccctggccccagctgattcgaaaaaaaaaaaaaaaaaaaaaaaaaaaaaaaaaaaaaaaaaaaaaaaaaaaaaaaaaaaaaaaaaaaaaaaaaaaaaaaaaaaaaaaaaaaaaaaaaaaaaaaaaaaaaaaaaaaaaaaa

SEQ ID NO: 10 - RNA, 4295 nt, synthetic construct
  misc_feature 1..4295: note = ETH031T30: C terminal EGFP tag-CCDC40 - codon optimized sequence encoding a functional version of a human CCDC40 protein
  source 1..4295: mol_type = other RNA
gggagacgccaccatggctgaacctggcggagccgccggaagatcccaccctgaagatggctctgccagcgagggcgagaaagagggcaacaacgagagccacatggtgtcccccccagagaaggacgacggccagaaaggcgaagaggccgtgggctctaccgagcaccctgaggaagtgaccacacaggccgaggccgccattgaagagggcgaggtggaaacagagggcgaagccgctgtggaaggcgaagaggaagccgtgtcttacggcgacgccgagagcgaggaagagtactactacaccgagacaagcagccccgagggccagatctctgccgccgataccacctacccctacttcagcccccctcaggaactgcctggggaagaggcctacgatagcgtgtccggcgaagctggcctgcagggctttcagcaggaagccacaggccctcccgagagccgggaaagaagagtgacaagccccgagcctagccacggcgtgctgggaccatctgagcagatgggccaagtgacctctggccctgctgtgggcagactgacaggcagcacagaggaacctcagggccaggtgctgcctatgggagtgcagcaccggttcagactgagccacggcagcgacatcgagagcagcgacctggaagagttcgtcagccaggaacccgtgatccctcctggcgtgccagatgcccatcccagggaaggcgatctgcccgtgttccaggaccagatccagcagccctctaccgaagagggggctatggccgagagagtggaaagcgagggctccgacgaagaagccgaggacgagggatctcagctggtggtgctggaccccgaccaccctctgatggtgcggtttcaggccgccctgaagaactacctgaaccggcagatcgagaagctgaaactggacctgcaggaactggtggtggccacaaagcagagcagagcccagagacaggaactgggcgtgaacctgtacgaggtgcagcagcatctggtgcatctgcagaagctgctggaaaagagccacgaccggcacgccatggccagctctgagcgcagacagaaagaggaagaactgcaggccgccagagccctgtacaccaagacatgcgccgctgccaacgaggaacggaagaagctggctgccctgcagaccgagatggaaaacctggctctgcacctgttctacatgcagaatatcgaccaggacatgcgggacgacatcagagtgatgacccaggtcgtgaagaaggccgagacagagagaatccgggccgagattgagaagaaaaagcaggacctgtacgtggaccagctgaccaccagggcccagcagctggaagaggatatcgccctgttcgaggcccagtacctggcccaggccgaagatacccggatcctgagaaaggccgtgtccgaggcctgcaccgagatcgatgccatcagcgtggaaaagcggcggatcatgcagcagtgggccagcagcctcgtgggcatgaagcacagagatgaggcccaccgggccgtgctggaagctctgagaggctgtcagcaccaggccaagagcaccgacggcgagatcgaggcctacaagaaatccatcatgaaggaagaggaaaagaacgagaaactggccagcatcctgaacagaaccgaaaccgaggccaccctgctgcagaaactgaccacccagtgcctgaccaaacaggtggccctgcagtcccagttcaacacctacagactgaccctgcaggacaccgaggacgccctgagtcaggatcagctggaacagatgattctgaccgaggaactgcaggctatccggcaggccattcagggggagctggaactgcggagaaagaccgacgccgccatcagagagaagctgcaggaacacatgaccagcaacaagaccaccaagtacttcaaccagctgattctgcgcctgcagaaagaaaagaccaacatgatgacacacctgagcaagatcaacggcgacattgcccagaccaccctggacatcacccacaccagcagcagactggacgcccaccagaaaaccctggtggaactggaccaggatgtgaagaaagtgaacgagctgatcaccaacagccagagcgagatcagccggcggaccatcctgatcgagagaaagcagggcctgatcaacttcctgaacaaacagctggaaagaatggtgtccgagctgggcggcgaggaagtgggacctctggaactggaaatcaagcggctgagcaagctgatcgacgagcacgacggcaaggccgtgcaggctcaagtgacatggctgcggctgcagcaggaaatggtcaaagtgacccaggaacaggaagaacagctggcctccctggacgccagcaagaaagaactgcacatcatggaacagaaaaagctgcgggtggaaagcaagatcgagcaggaaaaaaaagaacagaaagaaatcgagcaccacatgaaggacctggacaacgacctgaagaaactgaatatgctgatgaacaagaaccgctgctccagcgaagaactggaacagaacaacagagtgaccgagaacgagttcgtgcggagcctgaaggccagcgagcgggaaaccatcaagatgcaggacaagctgaaccagctgtccgaggaaaaagccacactgctgaaccagctggtggaagccgagcaccagatcatgctgtgggagaagaagatccagctggccaaagaaatgcggagcagcgtggacagcgagatcggccagaccgaaatcagagccatgaagggcgagatccaccggatgaaagtgcggctgggacagctgctgaaacagcaggaaaagatgatccgggccatggaactggccgtggccagacgggaaaccgtgacaacccaggctgagggccagcggaagatggacagaaaggccctgacccggaccgacttccaccacaagcagctggaactgaggcggaagatccgggacgtgcggaaggccaccgatgagtgcacaaagacagtgctggaactggaagagacacagcggaacgtgtcctccagcctgctggaaaaacaggaaaagctgagcgtgatccaggccgacttcgacaccctggaagctgacctgacaagactgggagccctgaaaagacagaacctgtccgagatcgtggcactgcagacccggctgaaacatctgcaggctgtgaaagagggacgctacgtgttcctgttcagatccaagcagtctctggtgctggaaagacagcggctggacaagcggctggcactgattgccaccatcctggatagagtgcgcgacgagtacccacagttccaggaagcactgcacaaggtgtcccagatgatcgccaacaagctggaatcccctggccccagcggcggagggggcagcgtgagcaagggcgaggagctgttcaccggggtggtgcccatcctggtcgagctggacggcgacgtaaacggccacaagttcagcgtgtccggcgagggcgagggcgatgccacctacggcaagctgaccctgaagttcatctgcaccaccggcaagctgcccgtgccctggcccaccctcgtgaccaccctgacctacggcgtgcagtgcttcagccgctaccccgaccacatgaagcagcacgacttcttcaagtccgccatgcccgaaggctacgtccaggagcgcaccatcttcttcaaggacgacggcaactacaagacccgcgccgaggtgaagttcgagggcgacaccctggtgaaccgcatcgagctgaagggcatcgacttcaaggaggacggcaacatcctggggcacaagctggagtacaactacaacagccacaacgtctatatcatggccgacaagcagaagaacggcatcaaggtgaacttcaagatccgccacaacatcgaggacggcagcgtgcagctcgccgaccactaccagcagaacacccccatcggcgacggccccgtgctgctgcccgacaaccactacctgagcacccagtccgccctgagcaaagaccccaacgagaagcgcgatcacatggtcctgctggagttcgtgaccgccgccgggatcactctcggcatggacgagctgtacaagtgattcgaaaaaaaaaaaaaaaaaaaaaaaaaaaaaaaaaaaaaaaaaaaaaaaaaaaaaaaaaaaaaaaaaaaaaaaaaaaaaaaaaaaaaaaaaaaaaaaaaaaaaaaaaaaaaaaaaaaaaaaa

SEQ ID NO: 11 - RNA, 5199 nt, synthetic construct
  misc_feature 1..5199: note = ETH031T26: N terminal HA Tag-CCDC40-T2A peptide-tdTomato with 5 and 3 CYBA UTRs - codon optimized sequence encoding a functional version of a human CCDC40 protein
  source 1..5199: mol_type = other RNA
gggagaccgcgcctagcagtgtcccagccgggttcgtgtcgccgccaccatgtacccctacgacgtgcccgactacgccggcggagggggcagcgctgaacctggcggagccgccggaagatcccaccctgaagatggctctgccagcgagggcgagaaagagggcaacaacgagagccacatggtgtcccccccagagaaggacgacggccagaaaggcgaagaggccgtgggctctaccgagcaccctgaggaagtgaccacacaggccgaggccgccattgaagagggcgaggtggaaacagagggcgaagccgctgtggaaggcgaagaggaagccgtgtcttacggcgacgccgagagcgaggaagagtactactacaccgagacaagcagccccgagggccagatctctgccgccgataccacctacccctacttcagcccccctcaggaactgcctggggaagaggcctacgatagcgtgtccggcgaagctggcctgcagggctttcagcaggaagccacaggccctcccgagagccgggaaagaagagtgacaagccccgagcctagccacggcgtgctgggaccatctgagcagatgggccaagtgacctctggccctgctgtgggcagactgacaggcagcacagaggaacctcagggccaggtgctgcctatgggagtgcagcaccggttcagactgagccacggcagcgacatcgagagcagcgacctggaagagttcgtcagccaggaacccgtgatccctcctggcgtgccagatgcccatcccagggaaggcgatctgcccgtgttccaggaccagatccagcagccctctaccgaagagggggctatggccgagagagtggaaagcgagggctccgacgaagaagccgaggacgagggatctcagctggtggtgctggaccccgaccaccctctgatggtgcggtttcaggccgccctgaagaactacctgaaccggcagatcgagaagctgaaactggacctgcaggaactggtggtggccacaaagcagagcagagcccagagacaggaactgggcgtgaacctgtacgaggtgcagcagcatctggtgcatctgcagaagctgctggaaaagagccacgaccggcacgccatggccagctctgagcgcagacagaaagaggaagaactgcaggccgccagagccctgtacaccaagacatgcgccgctgccaacgaggaacggaagaagctggctgccctgcagaccgagatggaaaacctggctctgcacctgttctacatgcagaatatcgaccaggacatgcgggacgacatcagagtgatgacccaggtcgtgaagaaggccgagacagagagaatccgggccgagattgagaagaaaaagcaggacctgtacgtggaccagctgaccaccagggcccagcagctggaagaggatatcgccctgttcgaggcccagtacctggcccaggccgaagatacccggatcctgagaaaggccgtgtccgaggcctgcaccgagatcgatgccatcagcgtggaaaagcggcggatcatgcagcagtgggccagcagcctcgtgggcatgaagcacagagatgaggcccaccgggccgtgctggaagctctgagaggctgtcagcaccaggccaagagcaccgacggcgagatcgaggcctacaagaaatccatcatgaaggaagaggaaaagaacgagaaactggccagcatcctgaacagaaccgaaaccgaggccaccctgctgcagaaactgaccacccagtgcctgaccaaacaggtggccctgcagtcccagttcaacacctacagactgaccctgcaggacaccgaggacgccctgagtcaggatcagctggaacagatgattctgaccgaggaactgcaggctatccggcaggccattcagggggagctggaactgcggagaaagaccgacgccgccatcagagagaagctgcaggaacacatgaccagcaacaagaccaccaagtacttcaaccagctgattctgcgcctgcagaaagaaaagaccaacatgatgacacacctgagcaagatcaacggcgacattgcccagaccaccctggacatcacccacaccagcagcagactggacgcccaccagaaaaccctggtggaactggaccaggatgtgaagaaagtgaacgagctgatcaccaacagccagagcgagatcagccggcggaccatcctgatcgagagaaagcagggcctgatcaacttcctgaacaaacagctggaaagaatggtgtccgagctgggcggcgaggaagtgggacctctggaactggaaatcaagcggctgagcaagctgatcgacgagcacgacggcaaggccgtgcaggctcaagtgacatggctgcggctgcagcaggaaatggtcaaagtgacccaggaacaggaagaacagctggcctccctggacgccagcaagaaagaactgcacatcatggaacagaaaaagctgcgggtggaaagcaagatcgagcaggaaaaaaaagaacagaaagaaatcgagcaccacatgaaggacctggacaacgacctgaagaaactgaatatgctgatgaacaagaaccgctgctccagcgaagaactggaacagaacaacagagtgaccgagaacgagttcgtgcggagcctgaaggccagcgagcgggaaaccatcaagatgcaggacaagctgaaccagctgtccgaggaaaaagccacactgctgaaccagctggtggaagccgagcaccagatcatgctgtgggagaagaagatccagctggccaaagaaatgcggagcagcgtggacagcgagatcggccagaccgaaatcagagccatgaagggcgagatccaccggatgaaagtgcggctgggacagctgctgaaacagcaggaaaagatgatccgggccatggaactggccgtggccagacgggaaaccgtgacaacccaggctgagggccagcggaagatggacagaaaggccctgacccggaccgacttccaccacaagcagctggaactgaggcggaagatccgggacgtgcggaaggccaccgatgagtgcacaaagacagtgctggaactggaagagacacagcggaacgtgtcctccagcctgctggaaaaacaggaaaagctgagcgtgatccaggccgacttcgacaccctggaagctgacctgacaagactgggagccctgaaaagacagaacctgtccgagatcgtggcactgcagacccggctgaaacatctgcaggctgtgaaagagggacgctacgtgttcctgttcagatccaagcagtctctggtgctggaaagacagcggctggacaagcggctggcactgattgccaccatcctggatagagtgcgcgacgagtacccacagttccaggaagcactgcacaaggtgtcccagatgatcgccaacaagctggaatcccctggccccagcggcagcggcgagggcagaggcagcctgctgacctgcggcgacgtggaggagaaccccggccccatggtgagcaagggcgaggaggtcatcaaagagttcatgcgcttcaaggtgcgcatggagggctccatgaacggccacgagttcgagatcgagggcgagggcgagggccgcccctacgagggcacccagaccgccaagctgaaggtgaccaagggcggccccctgcccttcgcctgggacatcctgtccccccagttcatgtacggctccaaggcgtacgtgaagcaccccgccgacatccccgattacaagaagctgtccttccccgagggcttcaagtgggagcgcgtgatgaacttcgaggacggcggtctggtgaccgtgacccaggactcctccctgcaggacggcacgctgatctacaaggtgaagatgcgcggcaccaacttcccccccgacggccccgtaatgcagaagaagaccatgggctgggaggcctccaccgagcgcctgtacccccgcgacggcgtgctgaagggcgagatccaccaggccctgaagctgaaggacggcggccactacctggtggagttcaagaccatctacatggccaagaagcccgtgcaactgcccggctactactacgtggacaccaagctggacatcacctcccacaacgaggactacaccatcgtggaacagtacgagcgctccgagggccgccaccacctgttcctggggcatggcaccggcagcaccggcagcggcagctccggcaccgcctcctccgaggacaacaacatggccgtcatcaaagagttcatgcgcttcaaggtgcgcatggagggctccatgaacggccacgagttcgagatcgagggcgagggcgagggccgcccctacgagggcacccagaccgccaagctgaaggtgaccaagggcggccccctgcccttcgcctgggacatcctgtccccccagttcatgtacggctccaaggcgtacgtgaagcaccccgccgacatccccgattacaagaagctgtccttccccgagggcttcaagtgggagcgcgtgatgaacttcgaggacggcggtctggtgaccgtgacccaggactcctccctgcaggacggcacgctgatctacaaggtgaagatgcgcggcaccaacttcccccccgacggccccgtaatgcagaagaagaccatgggctgggaggcctccaccgagcgcctgtacccccgcgacggcgtgctgaagggcgagatccaccaggccctgaagctgaaggacggcggccactacctggtggagttcaagaccatctacatggccaagaagcccgtgcaactgcccggctactactacgtggacaccaagctggacatcacctcccacaacgaggactacaccatcgtggaacagtacgagcgctccgagggccgccaccacctgttcctgtacggcatggacgagctgtacaagtgacctcgccccggacctgccctcccgccaggtgcacccacctgcaataaatgcagcgaagccgggattcgaaaaaaaaaaaaaaaaaaaaaaaaaaaaaaaaaaaaaaaaaaaaaaaaaaaaaaaaaaaaaaaaaaaaaaaaaaaaaaaaaaaaaaaaaaaaaaaaaaaaaaaaaaaaaaaaaaaaaaaa

SEQ ID NO: 12 - RNA, 2963 nt, synthetic construct
  misc_feature 1..2963: note = ETH047T02 (CCDC39 with Ethris minimal UTR) - codon optimized sequence encoding a functional version of a human CCDC39 protein
  source 1..2963: mol_type = other RNA
gggagacgccaccatgagcagcgagtttctggccgaactgcactgggaggacggcttcgctattcccgtggccaacgaggaaaacaagctgctggaagatcagctgagcaagctgaaggacgagagagcctctctgcaggacgagctgagagagtacgaggaacggatcaacagcatgaccagccacttcaagaacgtgaagcaagagctgagcatcacccagagcctgtgcaaggccagagagagagaaaccgagagcgaggaacacttcaaggctatcgcccagcgcgagctgggaagagtgaaggatgagatccagcggctggaaaacgagatggccagcatcctggaaaagaagtccgacaaagagaacggcatcttcaaggccacacagaagctggacggcctgaagtgccagatgaactgggatcagcaggccctggaagcctggctggaagagtctgcccacaaggattctgacgccctgacactgcagaagtacgcccagcaggacgacaacaagatccgggctctgaccctgcagctggaaagactgaccctggaatgcaaccagaagcggaagatcctggacaacgagctgaccgagacaatcagcgcccagctggaactggataaggccgctcaggacttcagaaagatccacaacgagcggcaagaactgatcaagcagtgggagaacaccatcgagcagatgcagaaacgcgacggcgacatcgacaactgcgccctggaactcgcccggatcaagcaagagacacgcgagaaagagaacctggtcaaagagaagatcaagttcctcgagtccgagatcggcaacaacaccgagttcgagaagcggatcagcgtggccgacagaaagctgctgaagtgcagaaccgcctaccaggaccacgagacaagccggattcagctcaagggcgagctggattctctgaaggccaccgtgaacagaaccagcagcgatctggaagccctgcggaagaacatcagcaagatcaagaaggacatccacgaggaaaccgccaggctgcagaaaacaaagaaccacaatgagatcatccagaccaagctgaaagagatcaccgaaaagaccatgagcgtggaagagaaggccacaaacctggaagatatgctcaaagaggaagagaaagacgtcaaagaggtggacgttcaactgaacctgattaagggcgtgctgttcaagaaggcccaagagctgcagaccgaaaccatgaaggaaaaggccgtcctgtctgagatcgagggcaccagatctagcctgaagcacctgaaccatcagctgcagaagctcgacttcgagacactgaagcagcaagagatcatgtacagccaggatttccacatccagcaggtcgagcggcggatgtctagactgaagggcgagatcaactccgaggaaaaacaggccctcgaggccaagatcgtggaactgagaaagagcctcgaagagaagaagtctacctgcggcctgctggaaacccagattaagaagctgcacaacgacctgtacttcatcaagaaagcccacagcaagaacagcgacgagaagcagagcctgatgaccaagatcaatgagctgaacctgttcatcgatcggagcgaaaaagagctggacaaggccaagggcttcaagcaggacctgatgatcgaggacaacctgctgaagctggaagtgaagcggaccagagagatgctgcacagcaaggccgaggaagtgctgtctctggaaaagcggaagcagcagctgtacaccgccatggaagagagaaccgaagagatcaaggtgcacaagaccatgctggcttcccagatcagatacgtggaccaagagcgcgagaacatctccaccgagtttagagagagactgtccaagatcgagaagctgaagaaccgctacgagatcctgaccgtcgtgatgctgcctcctgagggcgaagaggaaaagacccaggcctactacgtgatcaaggcagcccaagaaaaagaggaactccagagagaaggcgactgcctggacgccaagattaacaaggccgaaaaagaaatctacgccctcgagaacaccctgcaggtcctgaacagctgcaacaacaactacaagcagagcttcaagaaagtcacccctagctccgacgagtacgagctgaagattcagctggaagaacagaaaagagccgtggacgagaagtacagatacaagcagcggcagatcagagagctgcaagaggatatccagagcatggaaaacaccctggacgtgatcgagcacctggccaacaacgtgaaagagaagctgtccgagaaacaggcctacagctttcagctgtccaaagagacagaggaacagaagcccaaactggaacgcgtgaccaagcagtgcgccaagctgacaaaagagatccggctgctgaaagacaccaaggacgaaaccatggaagaacaagacatcaagctgcgcgagatgaagcagttccacaaagtgatcgacgagatgctggtggacatcattgaagagaacacagagatccgcatcatcctgcagacctattttcagcagagcggcctggaactgcctaccgcctctacaaagggcagcagacagagcagcagatcccctagccacacaagcctgagcgccagaagctctagaagcaccagcacctctaccagccagtccagcattaaggtgctggaactcaagttccccgccagctctagcctcgtgggaagcccttctagacctagcagcgcctctagcagctccagcaacgtgaagtccaagaaaagctccaagtgattcgaaaaaaaaaaaaaaaaaaaaaaaaaaaaaaaaaaaaaaaaaaaaaaaaaaaaaaaaaaaaaaaaaaaaaaaaaaaaaaaaaaaaaaaaaaaaaaaaaaaaaaaaaaaaaaaaaaaaaaaa

SEQ ID NO: 13 - RNA, 2964 nt, synthetic construct
  misc_feature 1..2964: note = RNA encoding for human CCDC39 sequence and contains TISU element as 5 UTR (ETH047T03) - codon optimized sequence encoding a functional version of a human CCDC39 protein
  source 1..2964: mol_type = other RNA
gggagactgccaagatgagcagcgagtttctggccgaactgcactgggaggacggcttcgctattcccgtggccaacgaggaaaacaagctgctggaagatcagctgagcaagctgaaggacgagagagcctctctgcaggacgagctgagagagtacgaggaacggatcaacagcatgaccagccacttcaagaacgtgaagcaagagctgagcatcacccagagcctgtgcaaggccagagagagagaaaccgagagcgaggaacacttcaaggctatcgcccagcgcgagctgggaagagtgaaggatgagatccagcggctggaaaacgagatggccagcatcctggaaaagaagtccgacaaagagaacggcatcttcaaggccacacagaagctggacggcctgaagtgccagatgaactgggatcagcaggccctggaagcctggctggaagagtctgcccacaaggattctgacgccctgacactgcagaagtacgcccagcaggacgacaacaagatccgggctctgaccctgcagctggaaagactgaccctggaatgcaaccagaagcggaagatcctggacaacgagctgaccgagacaatcagcgcccagctggaactggataaggccgctcaggacttcagaaagatccacaacgagcggcaagaactgatcaagcagtgggagaacaccatcgagcagatgcagaaacgcgacggcgacatcgacaactgcgccctggaactcgcccggatcaagcaagagacacgcgagaaagagaacctggtcaaagagaagatcaagttcctcgagtccgagatcggcaacaacaccgagttcgagaagcggatcagcgtggccgacagaaagctgctgaagtgcagaaccgcctaccaggaccacgagacaagccggattcagctcaagggcgagctggattctctgaaggccaccgtgaacagaaccagcagcgatctggaagccctgcggaagaacatcagcaagatcaagaaggacatccacgaggaaaccgccaggctgcagaaaacaaagaaccacaatgagatcatccagaccaagctgaaagagatcaccgaaaagaccatgagcgtggaagagaaggccacaaacctggaagatatgctcaaagaggaagagaaagacgtcaaagaggtggacgttcaactgaacctgattaagggcgtgctgttcaagaaggcccaagagctgcagaccgaaaccatgaaggaaaaggccgtcctgtctgagatcgagggcaccagatctagcctgaagcacctgaaccatcagctgcagaagctcgacttcgagacactgaagcagcaagagatcatgtacagccaggatttccacatccagcaggtcgagcggcggatgtctagactgaagggcgagatcaactccgaggaaaaacaggccctcgaggccaagatcgtggaactgagaaagagcctcgaagagaagaagtctacctgcggcctgctggaaacccagattaagaagctgcacaacgacctgtacttcatcaagaaagcccacagcaagaacagcgacgagaagcagagcctgatgaccaagatcaatgagctgaacctgttcatcgatcggagcgaaaaagagctggacaaggccaagggcttcaagcaggacctgatgatcgaggacaacctgctgaagctggaagtgaagcggaccagagagatgctgcacagcaaggccgaggaagtgctgtctctggaaaagcggaagcagcagctgtacaccgccatggaagagagaaccgaagagatcaaggtgcacaagaccatgctggcttcccagatcagatacgtggaccaagagcgcgagaacatctccaccgagtttagagagagactgtccaagatcgagaagctgaagaaccgctacgagatcctgaccgtcgtgatgctgcctcctgagggcgaagaggaaaagacccaggcctactacgtgatcaaggcagcccaagaaaaagaggaactccagagagaaggcgactgcctggacgccaagattaacaaggccgaaaaagaaatctacgccctcgagaacaccctgcaggtcctgaacagctgcaacaacaactacaagcagagcttcaagaaagtcacccctagctccgacgagtacgagctgaagattcagctggaagaacagaaaagagccgtggacgagaagtacagatacaagcagcggcagatcagagagctgcaagaggatatccagagcatggaaaacaccctggacgtgatcgagcacctggccaacaacgtgaaagagaagctgtccgagaaacaggcctacagctttcagctgtccaaagagacagaggaacagaagcccaaactggaacgcgtgaccaagcagtgcgccaagctgacaaaagagatccggctgctgaaagacaccaaggacgaaaccatggaagaacaagacatcaagctgcgcgagatgaagcagttccacaaagtgatcgacgagatgctggtggacatcattgaagagaacacagagatccgcatcatcctgcagacctattttcagcagagcggcctggaactgcctaccgcctctacaaagggcagcagacagagcagcagatcccctagccacacaagcctgagcgccagaagctctagaagcaccagcacctctaccagccagtccagcattaaggtgctggaactcaagttccccgccagctctagcctcgtgggaagcccttctagacctagcagcgcctctagcagctccagcaacgtgaagtccaagaaaagctccaagtgattcgaaaaaaaaaaaaaaaaaaaaaaaaaaaaaaaaaaaaaaaaaaaaaaaaaaaaaaaaaaaaaaaaaaaaaaaaaaaaaaaaaaaaaaaaaaaaaaaaaaaaaaaaaaaaaaaaaaaaaaaa

SEQ ID NO: 14 - RNA, 2993 nt, synthetic construct
  misc_feature 1..2993: note = ETH047T05: SP30; RNA encoding for human CCDC39 and containing random sequence of 30 nucleotides (SP30) which was used as 5 UTR - codon optimized sequence encoding a functional version of a human CCDC39 protein
  source 1..2993: mol_type = other RNA
gggagacattgaaatttatctcttgtgttgtggtcgcgccaccatgagcagcgagtttctggccgaactgcactgggaggacggcttcgctattcccgtggccaacgaggaaaacaagctgctggaagatcagctgagcaagctgaaggacgagagagcctctctgcaggacgagctgagagagtacgaggaacggatcaacagcatgaccagccacttcaagaacgtgaagcaagagctgagcatcacccagagcctgtgcaaggccagagagagagaaaccgagagcgaggaacacttcaaggctatcgcccagcgcgagctgggaagagtgaaggatgagatccagcggctggaaaacgagatggccagcatcctggaaaagaagtccgacaaagagaacggcatcttcaaggccacacagaagctggacggcctgaagtgccagatgaactgggatcagcaggccctggaagcctggctggaagagtctgcccacaaggattctgacgccctgacactgcagaagtacgcccagcaggacgacaacaagatccgggctctgaccctgcagctggaaagactgaccctggaatgcaaccagaagcggaagatcctggacaacgagctgaccgagacaatcagcgcccagctggaactggataaggccgctcaggacttcagaaagatccacaacgagcggcaagaactgatcaagcagtgggagaacaccatcgagcagatgcagaaacgcgacggcgacatcgacaactgcgccctggaactcgcccggatcaagcaagagacacgcgagaaagagaacctggtcaaagagaagatcaagttcctcgagtccgagatcggcaacaacaccgagttcgagaagcggatcagcgtggccgacagaaagctgctgaagtgcagaaccgcctaccaggaccacgagacaagccggattcagctcaagggcgagctggattctctgaaggccaccgtgaacagaaccagcagcgatctggaagccctgcggaagaacatcagcaagatcaagaaggacatccacgaggaaaccgccaggctgcagaaaacaaagaaccacaatgagatcatccagaccaagctgaaagagatcaccgaaaagaccatgagcgtggaagagaaggccacaaacctggaagatatgctcaaagaggaagagaaagacgtcaaagaggtggacgttcaactgaacctgattaagggcgtgctgttcaagaaggcccaagagctgcagaccgaaaccatgaaggaaaaggccgtcctgtctgagatcgagggcaccagatctagcctgaagcacctgaaccatcagctgcagaagctcgacttcgagacactgaagcagcaagagatcatgtacagccaggatttccacatccagcaggtcgagcggcggatgtctagactgaagggcgagatcaactccgaggaaaaacaggccctcgaggccaagatcgtggaactgagaaagagcctcgaagagaagaagtctacctgcggcctgctggaaacccagattaagaagctgcacaacgacctgtacttcatcaagaaagcccacagcaagaacagcgacgagaagcagagcctgatgaccaagatcaatgagctgaacctgttcatcgatcggagcgaaaaagagctggacaaggccaagggcttcaagcaggacctgatgatcgaggacaacctgctgaagctggaagtgaagcggaccagagagatgctgcacagcaaggccgaggaagtgctgtctctggaaaagcggaagcagcagctgtacaccgccatggaagagagaaccgaagagatcaaggtgcacaagaccatgctggcttcccagatcagatacgtggaccaagagcgcgagaacatctccaccgagtttagagagagactgtccaagatcgagaagctgaagaaccgctacgagatcctgaccgtcgtgatgctgcctcctgagggcgaagaggaaaagacccaggcctactacgtgatcaaggcagcccaagaaaaagaggaactccagagagaaggcgactgcctggacgccaagattaacaaggccgaaaaagaaatctacgccctcgagaacaccctgcaggtcctgaacagctgcaacaacaactacaagcagagcttcaagaaagtcacccctagctccgacgagtacgagctgaagattcagctggaagaacagaaaagagccgtggacgagaagtacagatacaagcagcggcagatcagagagctgcaagaggatatccagagcatggaaaacaccctggacgtgatcgagcacctggccaacaacgtgaaagagaagctgtccgagaaacaggcctacagctttcagctgtccaaagagacagaggaacagaagcccaaactggaacgcgtgaccaagcagtgcgccaagctgacaaaagagatccggctgctgaaagacaccaaggacgaaaccatggaagaacaagacatcaagctgcgcgagatgaagcagttccacaaagtgatcgacgagatgctggtggacatcattgaagagaacacagagatccgcatcatcctgcagacctattttcagcagagcggcctggaactgcctaccgcctctacaaagggcagcagacagagcagcagatcccctagccacacaagcctgagcgccagaagctctagaagcaccagcacctctaccagccagtccagcattaaggtgctggaactcaagttccccgccagctctagcctcgtgggaagcccttctagacctagcagcgcctctagcagctccagcaacgtgaagtccaagaaaagctccaagtgattcgaaaaaaaaaaaaaaaaaaaaaaaaaaaaaaaaaaaaaaaaaaaaaaaaaaaaaaaaaaaaaaaaaaaaaaaaaaaaaaaaaaaaaaaaaaaaaaaaaaaaaaaaaaaaaaaaaaaaaaaa